European Patent Application EP 4 726 031 A1, published April 15, 2026. Title: CLL1-CAR-T细胞及其制备方法与应用. Applicant: 浙江康佰裕生物科技有限公司. Application CN. The sequence listing filed with the application follows.

SEQUENCE LISTING (2 sequences)

SEQ ID NO: 1 - protein, 378 aa, synthetic construct
MALPVTALLLPLALLLHAARPDVQLQESGGGLVQPGGSLRLSCAASGFTFGDYDMTWVRQAPGKGPEWVSAINSGGGSTYYADSVKGRFTISRDNAKNTLYLQMNSLKPEDTAVYYCATIDRLSTVVAGTYQPSDEYDYWGQGTQVTVSSTTTPAPRPPTPAPTIASQPLSLRPEACRPAAGGAVHTRGLDFACDIYIWAPLAGTCGVLLLSLVITLYCRFSVVKRGRKKLLYIFKQPFMRPVQTTQEEDGCSCRFPEEEEGGCELRVKFSRSADAPAYQQGQNQLYNELNLGRREEYDVLDKRRGRDPEMGGKPRRKNPQEGLYNELQKDKMAEAYSEIGMKGERRRGKGHDGLYQGLSTATKDTYDALHMQALPPR

SEQ ID NO: 2 - DNA, 1134 bp, synthetic construct
  source 1..1134: mol_type = other DNA
atggctctgcctgtgaccgccctgctgctgcctctggctctgctgctgcacgccgctcggcctgatgtgcagctgcaggagtctggaggaggcttggtgcagcctgggggttctctgagactctcctgtgcagcctctggattcaccttcggagactatgacatgacctgggtccgccaggctccaggaaaggggcccgagtgggtctcagctattaatagtggcggtggtagcacatactatgcagactccgtgaagggccgattcaccatctccagagacaacgccaagaacacgctgtatctgcaaatgaacagcctgaaacctgaggacacggccgtgtattactgtgcaactatcgaccgccttagtacggtagtagctggtacgtaccagccgtccgatgagtatgactactggggccaggggacccaggtcaccgtctccagcactacaactccagcacccagaccccctacacctgctccaactatcgcaagtcagcccctgtcactgcgccctgaagcctgtcgccctgctgccgggggagctgtgcatactcggggactggactttgcctgtgatatctacatctgggcgcccttggccgggacttgtggggtccttctcctgtcactggttatcaccctttactgcaggttcagtgtcgtgaagagaggccggaagaagctgctgtacatcttcaagcagcctttcatgaggcccgtgcagactacccaggaggaagatggatgcagctgtagattccctgaagaggaggaaggaggctgtgagctgagagtgaagttctcccgaagcgcagatgccccagcctatcagcagggacagaatcagctgtacaacgagctgaacctgggaagacgggaggaatacgatgtgctggacaaaaggcggggcagagatcctgagatgggcggcaaaccaagacggaagaacccccaggaaggtctgtataatgagctgcagaaagacaagatggctgaggcctactcagaaatcgggatgaagggcgaaagaaggagaggaaaaggccacgacggactgtaccaggggctgagtacagcaacaaaagacacctatgacgctctgcacatgcaggctctgccaccaaga